European Patent Specification EP 3 595 725 B1, published May 3, 2023. Title: Combination Therapies for the Treatment of Breast Cancer. Applicant: Eisai R&D Management Co., Ltd. Karr, Craig Rioux, Nathalie Korpal, Manav Smith, Peter. The sequence listing filed with the application follows.

SEQUENCE LISTING (2 sequences)

SEQ ID NO: 1 - DNA, 39 bp, Homo sapiens
aagaacgtggtgcccctctctgacctgctgctggagatg

SEQ ID NO: 2 - DNA, 39 bp, Homo sapiens
catctccagcagcaggtcagagaggggcaccacgttctt